European Patent Specification EP 3 344 072 B1, published March 8, 2023. Title: METHODS AND COMPOSITIONS FOR DETECTING RISK OF CANCER RELAPSE. Applicant: Memorial Sloan-Kettering Cancer Center. The sequence listing filed with the application follows.

SEQUENCE LISTING (17 sequences)

SEQ ID NO: 1 - DNA, 1484 bp, Eubacterium limosum
agagtttgatcctggctcaggacgaacgctggcggtatgcttaacacatgcaagtcgaacgagaaggttttgatggatccttcgggtgacattagaactggaaagtggcgaacgggtgagtaacgcgtgggtaacctgccctatggaaaggaatagcctcgggaaactgggagtaaagccttatattatggttttgtcgcatggcaagatcatgaaaactccggtgccataggatggacccgcgtcccattagctagttggtgagataacagcccaccaaggcgacgatgggtaaccggtctgagagggcgaacggtcacactggaactgagacacggtccagactcctacgggaggcagcagtggggaatattgcgcaatgggggcaaccctgacgcagcaataccgcgtgagtgaagaaggttttcggatcgtaaagctctgttattggggaagaagaatgacggtacccaatgaggaagtcccggctaactacgtgccagcagccgcggtaatacgtaggggacaagcgttgtccggaatgactgggcgtaaagggcgcgtaggcggtctattaagtctgatgtgaaaggtaccggctcaaccggtgaagtgcattggaaactggtagacttgagtattggagaggcaagtggaattcctagtgtagcggtgaaatgcgtagatattaggaggaacaccagtggcgaaggcggcttgctggacaaatactgacgctgaggtgcgaaagcgtggggagcgaacaggattagataccctggtagtccacgccgtaaacgatgaatgctaggtgttggggaaactcagtgccgcagttaacacaataagcattccgcctggggagtacgaccgcaaggttgaaactcaaaggaattgacggggacccgcacaagcagcggagcatgtggtttaattcgaagcaacgcgaagaaccttaccaggtcttgacatcctctgacgagcctagagataggaagtttccttcgggaacagagagacaggtggtgcatggttgtcgtcagctcgtgtcgtgagatgttgggttaagtcccgcaacgagcgcaacccctgcctttagttgccagcattaagttgggcactctagagggactgccgtagacaatacggaggaaggtggggacgacgtcaaatcatcatgccccttatgacctgggctacacacgtgctacaatggtctgaacagagggccgcgaagccgcgaggtgaagcaaatcccttaaaacagatcccagttcggattgcaggctgcaactcgcctgcatgaagttggagttgctagtaatcgcggatcagaatgccgcggtgaatgcgttcccgggtcttgtacacaccgcccgtcacaccacgagagttggcaacacccgaagcctgtgagagaaccgcaaggactcagcagtcgaaggtggggctagtaattggggtgaagtcgtaacaaggtaacc

SEQ ID NO: 2 - DNA, 1393 bp, Peptococcus niger
gcctaatacatgcaagtcgaacggacgaggaaagagacctcttcggagtgacctttcccgagttagtggcggatgggtgagtaacgcgtgagtgacctgcccagcagtggggaataacagtgagaaatcattgctaataccgcatatcttacaagtgcttcatggtacctgtaagaaagacggccttcgtgctgtcgctgttggatggactcgcgtctgattagccagttggtggggtaacggcctaccaaagcaatgatcagtagccggcctgagagggtgaacggccacattgggactgagacacggcccaaactcctacgggaggcagcagtggggaatcttccgcaatgggcgcaagcctgacggagcaatgccgcgtgagtgaagaaggccttcgggttgtaaaactctgtcctcatccaagagaggggaaggtagtaactgacctttccaggacggtagatgaggaggaagccccggctaactatgtgccagcagccgcggtaaaacatagggggcaagcgttgtccggaatcactgggcgtaaagggcgcgcaggcggtctgttaagtcagatgtgaaaggttagggctcaaccctgaacgtgcatctgatactggcagacttgagtatggaagaggtaagtggaattcctagtgtagcggtgaaatgcgtagatattaggaggaacaccagtggcgaaggcgacttactgggccataactgacgctgaggcgcgaaagcgtggggagcaaacaggattagataccctggtagtccacgccgtaaacgatgggtactaggtgtcggaggtttcaagaccgtcggtgccgcagttaacacaataagtaccccgcctggggagtacggtcgcaagactgaaactcaaaggaattgacgggggcccgcacaagcggtggagcatgtggtttaattcgacgcaacgcgaagaaccttaccaagacttgacatcctgctgccgagtgatgtaatgtcacttttccttcgggacagcagagacaggtggtgcatggttgtcgtcagctcgtgtcgtgagatgttgggttaagtcccgcaacgagcgcaacccttgtcgtcagttgccatcattaagttgggcactctgacgagactgccgcagacaatgcggaggaaggtggggatgacgtcaaatcatcatgccccttatgtcttgggctacacacgtgctacaatggtcggtacagagggcagcgaaggagcgatccggagccaatctcacaaagccgatcccagttcggattgcaggctgcaactcgcctgcatgaagtcggaatgcgtagtaatcgcaggtcagcatactgcggtgaatacgttcccgggccttgtacacaccgcccgtcacaccacg

SEQ ID NO: 3 - DNA, 1462 bp, Anaerofustis stercorihominis
tggcggcgtgcttaacacatgcaagtcgaacgagaaacttataaatgatccttcgggtgaatctataagcggacagtggcgaacgggtgagtaacgcgtaggtaaccaacctcatgcagggggatagcccagggaaacttggattaaacccgcataagaccacagcaccgcatggtgcaggggtaaaaactccggtggcatgagacggacctgcgtcttattaggtagttggtgaggtaacggctcaccaagccaacgatgagtagccgacctgagagggtgatcggccacattgggactgagacacggcccagactcctacgggaggcagcagtggggaatattgcgcaatgggggaaaccctgacgcagcaacgccgcgtgagcgatgaaggttttcggatcgtaaagctctgtctttggggaagataatgacggtacccaaggaggaagctccggctaactacgtgccagcagccgcggtaatacgtagggagcaagcgttgtccggattcactgggcgtaaagagcacgtaggcggttaattaagtcaggtgtgaaagttttcggctcaaccggaaaagtgcacttgaaactggataacttgagtatcggagaggtaagcggaattcctagtgtagcggtgaaatgcgtagagattaggaagaacaccggtggcgaaggcggcttactggacgataactgacgctgaggtgcgaaagcgtggggagcgaacaggattagataccctggtagtccacgccgtaaacgatgaatactaggtgttggggtaactcagtgccgcagttaacacattaagtattccgcctggggagtacgctcgcaagagtgaaactcaaaggaattgacgggggcccgcacaagcagcggagcatgtggtttaattcgaagcaacgcgaagaaccttaccaggtcttgacatcccttgaccgcctaagagattaggctttccttcgggacaaggagacaggtggtgcatggttgtcgtcagctcgtgtcgtgagatgttgggttaagtcccgcaacgagcgcaacccttatgtttagttactaacattcagttgaggactctagacagactgcccttgaaagagggaggaaggtggggacgacgtcaaatcatcatgccccttacgacctgggctacacacgtgctacaatggtctgtacagagggttgcgaagcagtgatgctaagctaatctcaaaaagcagatctcagttcggattgcaggctgcaactcgcctgcatgaagtcggagttgctagtaatcgcgaatcagaatgtcgcggtgaatgcgttcccgggccttgtacacaccgcccgtcacaccacgagagttggtaacacccgaagccagtgagctaaccattaggaggcagctgtcgaaggtgggatcagtaattggggtgaagtcgtaacaaggtagccgtatcggaagg

SEQ ID NO: 4 - DNA, 1510 bp, Saccharofermentans acetigenes
ttgatcctggctcaggatgaacgctggcggcgtgcctaacacatgcaagtcgagcggagatgagaagagtacttgtacgaatttcatcttagcggcggacgggtgagtaatgcgtgaggaacctgcctttcactggggaataacatcgagaaatcggtgctaataccgcataaagtcgcgagatcgcatggttttgcgaccaaaggagcaatccggtgaaagatggactcacgtccgattaggtagttggtgaggtaacggcccaccaagcctacgatcggtagccgaactgagaggttgatcggccacattgggactgagacacggcccagactcctacgggaggcagcagtggggaatattgggcaatgggcgaaagcctgacccagcaacgccgcgtgaaggaagaaggtcttcggattgtaaacttctttgatcagggacgaaagaaatgacggtacctgaagaacaagccacggctaactacgtgccagcagccgcggtaatacgtaggtggcaagcgttatccggatttactgggtgtaaagggcgtgtaggcggttctgcaagtcagatgtgaaattcccgggcttaacccgggcgctgcatctgaaactgcaggacttgagtactggagaggatagtggaattcctagtgtagcggtaaaatgcgtagatattaggaggaacaccagtggcgaaggcggctatctggacagtaactgacgctgaggcgcgaaagcgtggggagcaaacaggattagataccctggtagtccacgccgtaaacgatgaatactaggtgtagggggtatcgactccccctgtgccgcagctaacgcaataagtattccacctggggagtacggccgcaaggttgaaactcaaaggaattgacgggggcccgcacaagcagtggattatgtggtttaattcgaagcaacgcgaagaaccttaccaggacttgacatcccttgaccggcatagagatatgcctttccttcgggacaaggagagcaggtggtgcatggttgtcgtcagctcgtgtcgtgagatgttgggttaagtcccgcaacgagcgcaacccctattgccagttgccatcattcagttgggaactctggcgatactgccgtggacaacacggaggaaggtggggacgacgtcaaatcatcatgccccttatgtcctgggctacacacgtaatacaatggcaacgacagagggcagctactccgcgaggacaagcgaatccctaaacgttgtctcagttcggattgcaggctgcaactcgcctgcatgaagtcggaattgctagtaatggcaggtcagcatactgccgtgaatacgttcccgggccttgtacacaccgcccgtcacaccatgagagtctgcaatacccgaagtcagtagtctaaccgcaagggggacgctgccgaaggtagggccgataattggggtgaagtcgtaacaaggtagccgtatcggaaggtgcggctggatcacctcc

SEQ ID NO: 5 - DNA, 1438 bp, Armatimonas rosea
gacgaacgctgcggcgtgcctaagaaatgcaagtcgaacggacagtggcttcggttactgttagtggcgaacggtcgcgtaacacgtaagaaacctgcctcgaagcgggggacaacagtccgaaaggactgctaataccgcatgtggccagtcgggggcatccccgattgtctaaagatttatcacttcgagatggtcttgcggcctatcagctagttggtggggtaacggcctaccaaggcgacgacgggtagctggtctgagaggacgatcagccggattgggactgagatacggcccagactcctacggggggcagcaattaggaatcttgcacaatgggcgaaagcctgatgcagcgacgccgcgtgaaggatgaaggttctcggatcgtaaacttcttttaagtgggaagaaatttgacggtaccacttgaataagccccggctaactacgtgccagcagccgcggtaatacgtagggggcgagcgttgtccgaagttactgggcgtaaagcgcgcgtaggcggtttcttaagtctggggtgaaaggttcaacgctcaacgtgaacagtgccttggatactgggagacttgagttagggagagggtagtagaattcctggtgtagcggtgaaatgcgtagatatcaggaggaataccaatggcgaaggcagctacctggcctataactgacgctgaggtgcgaaagcgtggggagcaaacgggattagataccccggtagtccacgccctaaacgatgagtgctagatgtaagaggtatcgacccctcttgtgtcgtcgctaacgcattaagcactccgcctggggagtacggccgcaaggttgaaactcaaaggaattgacgggggcccgcacaagcggtggagcatgtggattaattcgtcactaaccgaagaaccttacccaggtttgacatcctaggaaccctgatgaaagttgggggtgctcgcaagagagcctagagacaggtgttgcatggctgtcgtcagctcgtgtcgtgagatgttgggttaagtcccgcaacgagcgcaaccctcaccgtatgttggcagcgtaaagtcggcaactcttacggaactgcccgtgcaagcgggaggaaggtggggatgacgtcaagtcggcatggcccttacgcctggggcttcacacatgctacaatgggtggcaacaaagggctgctaaaccgtgaggtcaagcaaatcccaaaaatccatcctcagttcggattgtaggctgcaactcgcctacatgaagccggaatcgctagtaaccgcaggtcagctaaactgcggtgaatacgttcccgggccttgtacacaccgcccgtcaagtcacctgaattgtctgcacccgaagccggtggccaaactcgcaagagatggagccgtctaaggtgtggggagtaagggggact

SEQ ID NO: 6 - DNA, 1480 bp, Pseudoramibacter alactolyticus
taagtcaaaaagaacagtttgatcatggctcaggacgaacgctggcggtatgcttaacacatgcaagtcgaacgagaagttttttattgaccttcgggggatataagagacagacagtggcgaacgggtgagtaacgcgtgggcaacctacctatcggagcgggatagcctcgagaaatcgggagtaaaaccgcataacacagcagaatcgcatgactttgctgtcaaaactccggtgccgatagatgggcccgcgtctgattagctagttggtaaggtaagggcttaccaaggcaacgatcagtagccggtctgagagggcgaacggccacactggaactgagacacggtccagactcctacgggaggcagcagtggggaatattgcgcaatgggggcaaccctgacgcagcaataccgcgtgagtgaagaaggttttcggatcgtaaagctctgttattggggaagaagcagtgacggtacccaatgaggaagtcccggctaactacgtgccagcagccgcggtaatacgtaggggacgagcgttgtccggaatcactgggcgtaaagggcgcgtaggcggttttataagtcagatgtgaaaggtaccggctcaaccggtgacgtgcatttgaaactgtaagacttgagtactgaagaggcaagcggaattcctagtgtagcggtgaaatgcgtagatattaggaagaacaccggtggcgaaggcggcttgctgggcagatactgacgctgaggtgcgaaagcgtggggagcgaacaggattagataccctggtagtccacgccgtaaacgatgaatactaggtgttggcgaataagtcagtgccggagttaacacaataagtattccgcctggggagtacgaccgcaaggttgaaactcaaaggaattgacggggacccgcacaagcagcggagcatgtggtttaattcgaagcaacgcgaagaaccttaccaggccttgacatcctctgagcgcaatagagatattgctttcccttcggagacagagagacaggtggtgcatggttgtcgtcagctcgtgtcgtgagatgttgggttaagtcccgcaacgagcgcaacccctgtcattagttgccatcattgagttgggcactctaatgagactgccgtagacaatacggaggaaggtggggacgacgtcaaatcatcatgccccttatggcctgggctacacacgtgctacaatggtctgaacaaagggaagcgaaggagcgattcggagcgaatctcataaaacagatcccagttcggattgcaggctgcaactcgcctgcatgaagatggagttgctagtaatcgcggatcagaatgtcgcggtgaatgcgttcccgggtcttgtacacaccgcccgtcacaccacgagagtcggtaacacccgaagccagtgagacaaccggaaggagtcagctgtcgaaggtgggatcggtaattggggtg

SEQ ID NO: 7 - DNA, 1483 bp, Finegoldia magna
agagtttgatcctggctcaggacgaacgctggcggcgtgcttaacacatgcaagtcgaacgggatttagtagacagaagcttcggtggaagattactaatgagagtggcgaacgggtgagtaacgcgtgagcaacctgcctatgacagtgggatagcctcgggaaaccgggattaataccgcataaaatcgtagaaacacatgttttaacggtcaaagatttatcggtcatagatgggctcgcgtctgattagctagttggtgagataacagcccaccaaggcgacgatcagtagccggtctgagaggatgaacggccacattggaactgagacacggtccaaactcctacgggaggcagcagtggggaatattgcacaatgggggaaaccctgatgcagcgacgccgcgtgaacgaagaaggtattcgtatcgtaaagttctgtcctatgggaagataatgacagtaccatagaagaaagctccggctaaatacgtgccagcagccgcggtaatacgtatggagcgagcgttgtccggaattattgggcgtaaagggtacgcaggcggtttaataagtcgaatgttaaagatcggggctcaaccccgtaaagcattggaaactgataaacttgagtagtggagaggaaagtggaattcctagtgtagtggtgaaatacgtagatattaggaggaataccagtagcgaaggcgactttctggacacaaactgacgctgaggtacgaaagcgtggggagcaaacaggattagataccctggtagtccacgccgtaaacgatgaatgctaggtgttgggggtcaaacctcggtgccgaagttaacacattaagcattccgcctggggagtacgcacgcaagtgtgaaactcaaaggaattgacggggacccgcacaagcagcggagcatgtggtttaattcgatgcaacgcgaagaaccttaccagggcttgacatgtgggtgaaaggtatagagatatacccctctctttatgagacatccatacaggtggtgcatggttgtcgtcagctcgtgtcgtgagatgttgggttaagtcccgcaacgagcgcaacccctatacttagttaccagcgagtaaagtcggggactctaagtagactgccgatgacaaatcggaggaaggtggggatgacgtcaaatcatcatgccctttatgtcctgggctacacacgtgctacaatggttggtacagagggaagctatatagtgatataatgcaaaactccaaagccaatcccagttcggattgtaggctgcaactcgcctacatgaagtcggagttgctagtaatcgcggatcagaatgtcgcggtgaatgcgttcccgggtcttgtacacaccgcccgtcacaccatgggagttgataatacccgaagcctgtgacctaattgaggagcagtcgaaggtaggattgatgactggggtgaagtcgtaacaaggtaacc

SEQ ID NO: 8 - DNA, 1362 bp, Murdochiella asaccharolytica
  misc_feature (643)..(643): n is a, c, g, or t
aacgagaatgtactgacggatccttagggtgaagatagtacaggacagtggcggatgggtgagtaacgcgtaagaaacctgcctttcacaccgggatagcagctggaaacggctattaataccggatgacactttttccccgcatgaggaagaggttaaagaatttcggtgaaagatggtcttgcgtctgattagctagttggtggggtaacggcctaccaaggcgacgatcagtagccggcctgagagggtgtacggccacattgggactgagacacggcccaaactcctacgggaggcagcagtggggaattttgcacaatggaggaaactctgatgcagcgacgccgcgtgaacgaagaaggtcttcggattgtaaagttctgtcctgggtgaagataatgacggtaactcaggaggaagccccggctaactacgtgccagcagccgcggtaatacgtagggggcgagcgttgttcggaattattgggcgtaaagggtacgtaggcggtttgttaagtttggcgttaaatcacggggctcaaccccgttcagcgttgaaaactggcaaacttgagtagtagaggggacagtggaattcctagtgtagcggtgaaatgcgtagagattaggaagaataccngtggcgaaggcgactgtctggatacatactgacgctcaggtacgaaagcgtggggagcaaacaggattagataccctggtagtccacgccctaaacgatgagtgctaggtgtcgggtgtcaaagctcggtgccgccgttaacacattaagcactccgcctggggagtacgcacgcaagtgtgaaactcaaatgaattgacggagacccgcacaagtagcggagcatgtggtttaattcgaagcaacgcgaagaaccttaccagggcttgacataacagtgacgggttaagagattaaccgttcccttcggggacactgctacaggtggtgcatggttgtcgtcagctcgtgtcgtgagatgttgggttaagtcccgcaacgagcgcaacccttgtcgttagttgccagcattgagttggggactctagcgagactgccggtgataaaccggaggaaggtggggatgacgtcaaatcatcatgccctttatgtcctgggctacacacgtgctacaatggccgaaaacagcgtgaagcaacctcgtgagagcaagcgaaccacgaaaagtcggtctcagttcggactgtaggctgcaactcgcctacacgaagtcggagttactagtaatcgcgaatcagcatgtcgcggtgaatgcgttcccgggtcttgtacacaccgcccgtcacaccatggaagttggtaatacccgaagccgctga

SEQ ID NO: 9 - DNA, 1489 bp, Levyella massiliensis
tagagtttgatcctggctcaggataaacgctggcggcgtgcgtaacacatgcaagtcgaacgagaatgtgctgacggatccttagggtgaagatagcacaggacagtggcggatgggtgagtaacgcgtaagaaacctgcctttcacaccgggatagcagctggaaacggctattaataccggatgacactttttccccgcatgaggaagaggttaaagaatttcggtgaaagatggtcttgcgtctgattagctagttggtggggtaacggcctaccaaggcgacgatcagtagccggcctgagagggtgtacggccacattgggactgagacacggcccaaactcctacgggaggcagcagtggggaattttgcacaatggaggaaactctgatgcagcgacgccgcgtgaacgaagaaggtcttcggattgtaaagttctgtcctgggtgaagataatgacggtaactcaggaggaagccccggctaactacgtgccagcagccgcggtaatacgtagggggcgagcgttgttcggaattattgggcgtaaagggtacgtaggcggtttgttaagtttggcgttaaatcacggggctcaaccccgttcagcgttgaaaactggcaaacttgagtagtagaggggacagtggaattcctagtgtagcggtgaaatgcgtagagattaggaagaataccggtggcgaaggcgactgtctggatacatactgacgctcaggtacgaaagcgtggggagcaaacaggattagataccctggtagtccacgccctaaacgatgagtgctaggtgtcgggtgtcaaagcccggtgccgccgttaacacattaagcactccgcctggggagtacgcacgcaagtgtgaaactcaaaggaattgacggggacccgcacaagtagcggagcatgtggtttaattcgaagcaacgcgaagaaccttaccagggcttgacataacagtgacgggttaagagattaaccgttcccttcggggacactgctacaggtggtgcatggttgtcgtcagctcgtgtcgtgagatgttgggttaagtcccgcaacgagcgcaacccttgtcgttagttgccagcattaagttggggactctagcgagactgccggtgataaaccggaggaaggtggggatgacgtcaaatcatcatgccctttatgtcctgggctacacacgtgctacaatggccgaaaacagcgtgaagcaacctcgtgagagcaagcgaaccacgaaaagtcggtctcagttcggactgtaggctgcaactcgcctacacgaagtcggagttactagtaatcgcgaatcagcatgtcgcggtgaatgcgttcccgggtcttgtacacaccgcccgtcacaccatggaagttggtaatacccgaagccgctgagcgaacctatgacgcaggcgtcgaaggtaggatcaatgactggggtgaagtcgtaacaaggtagccgta

SEQ ID NO: 10 - DNA, 1357 bp, Gallicola barnesae
  misc_feature (20)..(20): n is a, c, g, or t
  misc_feature (55)..(55): n is a, c, g, or t
  misc_feature (493)..(496): n is a, c, g, or t
  misc_feature (888)..(895): n is a, c, g, or t
cgaacgctggcggcgtgatnaaaacatgcaagtcgaacgatcacccttccatttntctattcggagagattgaggagcgggttaggggagaggggttgaataacgtgtgagccaccctgtctaaacaaggggatagcctcgggactccgggatttattccgtatgagaccccgccttcccatgtagaagaggttcaaagattttatcggtttaagatgggctcgcgtctgattagctagttggtgagataaaagcccaccaagtcaacgatcagtaaccggcttgagagagtgaacggtcacattggacactgagacacggtccaaactcctcagggaggcagcagtggggaatattgcacaatgggggaaaccctgatgcagcgacgccgcgtgagcgatgaaggaattcgtttcgtaaagctctgtcctaggggaagataatgacagtacccttggaggaagccccggctaaatacgtgcgcagcagccgnnnnttacgtatggggcgagcgttgtccggaattattgggcgtaaagggtacgtaggcggtttcataagtcagatgtaaaagcgtggggctcaaccccataaagcatttgaaactgtggaacttgagtagtggagaggaaagtggaattcctagtgtagcggtgaaatgcgtagatattaggaggaataccagtggcgaaggcgactttctggacacaaactgacgctgaggtacgaaagcatggggagcacacaggattagataccctggtagtccatgccgtaaacgatgaatgctaggtgtcgggggtcaaacctcggtgccgcagttaacacagtaagcattccgcctggggagtacggtggcaacactgaaactcaatggatcaaatgaannnnnnnnggcccgcgcaagcagcggagcatgtggtttatttcgatgcaacgcgaagaaccttaccaggacttgacatatagatgaaagatctagagatagatccctctcttcggagacagctatacaggtggtgcatggttgtcgtcagctcgtgtcgtgagatgttgggttaagtcccgcaacgagcgcaccccctatagctagttaccagcacttcgggtggggactctagttagactgccgatgataaatcggaggaaggtggggatgacgtcaaatcatcatgccctttatgtcctgggctacacacgtgctacaatggtcggtacagagggcagcgagactgtgaagttaagcgaatctcagaaagccgaccccagttcggattgcaggcttgcaactcgcctgcatgaagtcggagttggtagtaatcgcagatcagaatgctgcggtgaatgcttgccgctc

SEQ ID NO: 11 - DNA, 1438 bp, Eubacterium brachy
gatgaacgctggcggcgtgcttaacacatgcaagtcgagcgagaagttttgaaaagattcttcggatgaaatttaaaatggaaagcggcggacgggtgagtaacgcgtaggcaaccatacaaagggatagcatttggaaacgaatattaataccttatgaaacttaactagtgcatgctaggtaggtcaaagatttatcggtatgggatgggcctgcgtctgactgcccttagctagttggtgaggtaacggctcaccaaggcgacgatcagtagccgacctgagagggtgaacggccacattggaactgagacacggtccaaactcctacgggaggcagcagtggggaatattgcacaatgggggaaaccctgatgcagcaacgccgcgtgaacgatgaaggcctttgggtcgtaaagttctgttctaggtgatgaaaactgacagtaacctaggagaaagccccggctaactccgtgccagcagccgcggtaatactggagggggcaagcgttatccggaattattgggcgtaaagggtacgtaggtggccttttaagcgtagggtataaggcaatggctcaaccattgttcgccctatgaactggaaggcttgagtgcaggagaggaaagcggaattcctagtgtagcggtggaatgcatagatattaggaggaacatcagcggcgaaggcggctttctggactgcaactgacactgaggtacgaaagcgtggggagcaaacaggattagataccctggtagtccacgccgtaaacgatgagcactaggtgtcggggtcgtaaggcttcggtgccgtagttaacgcattaagtgctccgcctggggagtacgcacgcaagtgtgaaactcaaaggaattgacggggacccgcacaagcagcggagcatgtggtttaattcgaagcaacgcgagaaccttaccaggacttgacatccttctgaccggtctttaataggacctttcttttgacagaagagacaggtggtgcatggttgtcgtcagctcgtgtcgtgagatgttgggttaagtcccgcaacgagcgcaacccttgtcattagttgccatcattaagttgggcactctagtgagactgccggggacaactcggaggaaggtggggatgacgtcaaatcatcatgccccttatgttctgggctacacacgtgctacaatggctggtacaaagagaagcaagaccgcaaggtggagcaaagctcaaaaaccagccccagttcggattgtaggctgaaactcgcctacatgaagtcggagttgctagtaatcgcagatcagaatgctgcggtgaatgcgttcccgggtcttgtacacaccgcccgtcacaccatggaagttgggggcgcccaaagttggcagataaatatgctacctaaggtgaaaccaatgactggggtga

SEQ ID NO: 12 - DNA, 1487 bp, Parvimonas micra
agagtttgatcctggctcaggacgaacgctggcggcgtgcttaacacatgcaagtcgaacgtgatttttgtggaaattctttcgggaatggaaatgaaatgaaagtggcgaacgggtgagtaacacgtgagcaacctaccttacacagggggatagccgttggaaacgacgattaataccgcatgagaccacagaatcgcatgatataggggtcaaagatttatcggtgtaagaagggctcgcgtctgattagctagttggaagggtaaaggcctaccaaggcgacgatcagtagccggtctgagaggatgaacggccacattggaactgagacacggtccaaactcctacgggaggcagcagtggggaatattgcacaatggggggaaccctgatgcagcgacgccgcgtgagcgaagaaggttttcgaatcgtaaagctctgtcctatgagaagataatgacggtatcataggaggaagccccggctaaatacgtgccagcagccgcggtaatacgtatggggcgagcgttgtccggaattattgggcgtaaagggtacgtaggcggttttttaagtcaggtgtgaaagcgtgaggcttaacctcattaagcacttgaaactggaagacttgagtgaaggagaggaaagtggaattcctagtgtagcggtgaaatgcgtagatattaggaggaataccggtggcgaaggcgactttctggacttttactgacgctcaggtacgaaagcgtggggagcaaacaggattagataccctggtagtccacgccgtaaacgatgaatgctaggtgttgggagtcaaatctcggtgccgaagttaacacattaagcattccgcctggggagtacggtggcaacactgaaactcaaaggaattgacggggacccgcacaagcagcggagcatgtggtttaattcgaagcaacgcgaagaaccttaccaaggcttgacatatagttgagttattgagaaattgataagtccctcgggacaactatacaggtggtgcatggttgtcgtcagctcgtgtcgtgagatgttgggttaagtcccgcaacgagcgcaacccttatcttcagttgccagcacgtagaggtgggaactctggagagactgccgatgacaaatcggaggaaggtggggatgacgtcaaatcatcatgccctttatgtcttgggctacacacgtgctacaatggttggtacaacgagaagcgagatagagatgttaagcgaaactctaaaaaccaatctcagttcggattgtaggctgcaactcgcctacatgaagtcggagttgctagtaatcgcgaatcagaatgtcgcggtgaatgcgttcccgggtcttgtacacaccgcccgtcacaccatgggagttggcaatacccgaagccgccgatctaaccgcaaggaggaaggcgtcgaaggtagggttaatgactggggtgaagtcgtaacaaggtaacc

SEQ ID NO: 13 - DNA, 1478 bp, Streptococcus anginosus
gacgaacgctggcggcgtgcctaatacatgcaagtaggacgcacagtttataccgtagcttgctacaccatagactgtgagttgcgaacgggtgagtaacgcgtaggtaacctgcctattagagggggataactattggaaacgatagctaataccgcataacagtatgtaacacatgttagatgcttgaaagatgcaattgcatcgctagtagatggacctgcgttgtattagctagtaggtagggtaatggcctacctaggcgacgatacatagccgacctgagagggtgatcggccacactgggactgagacacggcccagactcctacgggaggcagcagtagggaatcttcggcaatggggggaaccctgaccgagcaacgccgcgtgagtgaagaaggttttcggatcgtaaagctctgttgttaaggaagaacgagtgtgagaatggaaagttcatactgtgacggtacttaaccagaaagggacggctaactacgtgccagcagccgcggtaatacgtaggtcccgagcgttgtccggatttattgggcgtaaagcgagcgcaggcggttagaaaagtctgaagtgaaaggcagtggctcaaccattgtaggctttggaaactgtttaacttgagtgcagaaggggagagtggaattccatgtgtagcggtgaaatgcgtagatatatggaggaacaccggtggcgaaagcggctctctggtctgtaactgacgctgaggctcgaaagcgtggggagcgaacaggattagataccctggtagtccacgccgtaaacgatgagtgctaggtgttgggtcctttccgggactcagtgccgcagctaacgcattaagcactccgcctggggagtacgaccgcaaggttgaaactcaaaggaattgacgggggcccgcacaagcggtggagcatgtggtttaattcgaagcaacgcgaagaaccttaccaggtcttgacatcccgatgctatttctagagataggaagtttcttcggaacatcggtgacaggtggtgcatggttgtcgtcagctcgtgtcgtgagatgttgggttaagtcccgcaacgagcgcaacccttattgttagttgccatcattaagttgggcactctagcgagactgccggtaataaaccggaggaaggtggggatgacgtcaaatcatcatgccccttatgacctgggctacacacgtgctacaatggctggtacaacgagtcgcaagccggtgacggcaagctaatctctgaaagccagtctcagttcggattgtaggctgcaactcgcctacatgaagtcggaatcgctagtaatcgcggatcagcacgccgcggtgaatacgttcccgggccttgtacacaccgcccgtcacaccacgagagtttgtaacacccgaagtcggtgaggtaaccgtaaggagccagccgcctaaggtgggatagatgattggggtg

SEQ ID NO: 14 - DNA, 1487 bp, Eubacterium biforme
  misc_feature (31)..(31): n is a, c, g, or t
  misc_feature (120)..(120): n is a, c, g, or t
  misc_feature (242)..(242): n is a, c, g, or t
  misc_feature (341)..(342): n is a, c, g, or t
  misc_feature (579)..(579): n is a, c, g, or t
  misc_feature (928)..(929): n is a, c, g, or t
  misc_feature (933)..(933): n is a, c, g, or t
  misc_feature (968)..(968): n is a, c, g, or t
  misc_feature (1229)..(1229): n is a, c, g, or t
  misc_feature (1385)..(1385): n is a, c, g, or t
caaatggagagtttgatcctggctcaggatnaacgctggcggcatgcctaatacatgcaagtcgaacgagaggaaggaaagcttgcttttctgaatctagtggcgaacgggtgagtaacncgtaggtaacctgcccatgtgcccgggataacttctggaaacggatgctaaaaccggataggtagcagacaagcatttgactgctattaaagtggctaaggccatgaacatggatggacctncggtgcattagctagttggtgaggtaacggcccaccaaggcgacgatgcatagccggcctgagagggcggacggccacattgggactgagacacggccnnaactcctacgggaggcagcagtagggaattttcgtcaatggggggaaccctgaacgagcaatgccgcgtgagtgaggaaggtcttcggatcgtaaagctctgttgtaagagaaaaacgacattcatagggaatgatgagtgagtgatggtatcttaccagaaagtcacggctaactacgtgccagcagccgcggtaatacgtaggtggcgagcgttatccggaatgattgggcgtanagggtgcgtaggtggcagaacaagtctggagtaaaaggtatgggctcaacccgtactggctctggaaactgttcagctagagaacagaagaggacggcggaactccatgtgtagcggtaaaatgcgtagatatatggaagaacaccggtggcgaaggcggccgtctggtctgttgctgacactgaagcacgaaagcgtggggagcaaataggattagataccctagtagtccacgccgtaaacgatgagaactaggtgttgggggaataactcagtgccgcagttaacgcaataagttctccgcctggggagtatgcacgcaagtgtgaaactcaaaggaattgacggnngccngcacaagcggtggagtatgtggtttaattcgaagnaacgcgaagaaccttaccaggccttgacatcccttgcagagrtatagagatatatccgaggttaacaaggagacaggtggtgcatggttgtcgtcagctcgtgtcgtgagatgttgggttaagtcccgcaacgagcgcaacccttgtgatatgttactaacattgagttgaggactcatatcagactgccggtgataaaccggaggaaggtggggatgacgtcaaatcatcatgccccttatggcctgggctacacacgtnctacaatggcgtctacaaagagcggcaagcctgtgaaggcaagcgaatctcataaaggacgtctcagttcggattgaagtctgcaacccgacttcatgaagctggaatcgctagtaatcgcgaatcagcatgtcgcggtgaatacgttctcgggcnttgtacacaccgcccgtcaaaccatgggagttggtaatgcccgaagccggtggcataacctttcgaggagtgagccgtcgaaggcaggaccgatgactgggg

SEQ ID NO: 15 - DNA, 1439 bp, Acidaminococcus intestini
gcggagacttatttcggtaagttcttagtggcgaacgggtgagtaacgcgtgggcaacctgccctccagttggggacaacattccgaaagggatgctaataccgaatgtgctccctcctccgcatggaggagggaggaaagatggcctctgcttgcaagctatcgctggaagatgggcccgcgtctgattagctagttggtggggtaacggctcaccaaggcgatgatcagtagccggtctgagaggatgaacggccacattgggactgagacacggcccaaactcctacgggaggcagcagtggggaatcttccgcaatggacgaaagtctgacggagcaacgccgcgtgagtgatgaaggtcttcggattgtaaaactctgttgttagggacgaaagcaccgtgttcgaacaggtcatggtgttgacggtacctaacgaggaagccacggctaactacgtgccagcagccgcggtaatacgtaggtggcaagcgttgtccggaattattgggcgtaaagagcatgtaggcgggcttttaagtctgacgtgaaaatgcggggcttaaccccgtatggcgttggatactggaagtcttgagtgcaggagaggaaaggggaattcccagtgtagcggtgaaatgcgtagatattgggaggaacaccagtggcgaaggcgcctttctggactgtgtctgacgctgagatgcgaaagccagggtagcaaacgggattagataccccggtagtcctggccgtaaacgatggatactaggtgtaggaggtatcgaccccttctgtgccggagttaacgcaataagtatcccgcctggggactacgatcgcaagattgaaactcaaaggaattgacgggggcccgcacaagcggtggagtatgtggtttaattcgacgcaacgcgaagaaccttaccaaggcttgacattgagtgaaagacctagagataggtccctcccttcggggacacgaaaacaggtggtgcatggctgtcgtcagctcgtgtcgtgagatgttgggttaagtcccgcaacgagcgcaacccctatcctatgttaccagcgcgtaatggcggggactcataggagactgccagggataacttggaggaaggcggggatgacgtcaagtcatcatgccccttatgtcttgggctacacacgtactacaatggtcggcaacaaagggcagcgaaaccgcgaggtggagcaaatcccagaaacccgaccccagttcggatcgtaggctgcaacccgcctacagtgaagttggaatcgctagtaatcgcaggtcagcatactgcggtgaatacgttcccgggccttgtacacaccgcccgtcacaccacgaaagttggtaacacccgaagccggtgagataaccttttaggagtcagctgtctaaggtggggccgatgattgggg

SEQ ID NO: 16 - DNA, 1493 bp, Clostridium glycyrrhizinilyticum
  misc_feature (207)..(207): n is a, c, g, or t
agagtttgatcctggctcaggatgaacgctggcggcgtgcttaacacatgcaagtcgaacgaagcactttaccggatttcttcggaatgaaagttttgtgactgagtggcggacgggtgagtaacgcgtgggtaacctgcctcatacagggggataacagttagaaatgactgctaataccgcataagaccacaggaccgcatggtncggtggtaaaaactccggtggtatgagatggacccgcgtctgattagctagttggtaaggtaacggcttaccaaggcgacgatcagtagccgacctgagagggtgaccggccacattgggactgagacacggcccaaactcctacgggaggcagcagtggggaatattgcacaatgggggaaaccctgatgcagcgacgccgcgtgagcgatgaagtatttcggtatgtaaagctctatcagcagggaagaattaggacggtacctgactaagaagcaccggctaaatacgtgccagcagccgcggtaatacgtatggtgcaagcgttatccggatttactgggtgtaaagggagcgtagacggagaggcaagtctgatgtgaaaacccggggctcaaccccgggactgcattggaaactgtttttctagagtgtcggagaggtaagtggaattcctagtgtagcggtgaaatgcgtagatattaggaggaacaccagtggcgaaggcggcttactggacgatgactgacgttgaggctcgaaagcgtggggagcaaacaggattagataccctggtagtccacgccgtaaacgatgactgctaggtgtcgggaggcaaagcctttcggtgccgcagcaaacgcaataagcagtccacctggggagtacgttcgcaagaatgaaactcaaaggaattgacggggacccgcacaagcggtggagcatgtggtttaattcgaagcaacgcgaagaaccttacctgcccttgacatccggctgaccggcgagtaatgtcgcctttccttcgggacagccgagacaggtggtgcatggttgtcgtcagctcgtgtcgtgagatgttgggttaagtcccgcaacgagcgcaacccttatctttagtagccagcatttcggatgggcactctagagagactgccagggataacctggaggaaggtggggatgacgtcaaatcatcatgccccttatgggcagggctacacacgtgctacaatggcgtaaacaaagggaggcaagcctgcgagggtgagcaaatcccaaaaataacgtctcagttcggattgtagtctgcaactcgactacatgaagctggaatcgctagtaatcgcgaatcagaatgtcgcggtgaatacgttcccgggtcttgtacacaccgcccgtcacaccatgggagttggtaacgcccgaagtcagtgacccaaccgtaaggagggagctgccgaaggtgggaccgataactggggtgaagtcgtaacaaggtaacc

SEQ ID NO: 17 - DNA, 1553 bp, Desulfosporosinus lacus
gatcctggctcaggacgaacgctggcggcgtgcctaacacatgcaagtcgaacggagaatttcaataagtttacttagagaagtttttagtggcggacgggtgagtaacgcgtgggtaacctacccataaagccgggacaacccttggaaacgagggctaataccggataatctttgatgttggcatcaaggttaaaggaaaggtggcctctgaagatgctaccgattatggatggacccgcgtctgattagctagttggtggggtaaaggcctaccaaggcgacgatcagtagccggcctgagagggtgaacggccacactgggactgagacacggcccagactcctacgggaggcagcagtggggaatcttccgcaatggacgaaagtctgacggagcaacgccgcgtgtatgatgaaggtcttcggattgtaaagtactgtctttggggaagaatgactgatttgaaaatattgagtcagtatgacggtacccaaggaggaagccccggctaactacgtgccagcagccgcggtaatacgtagggggcaagcgttgtccggaattattgggcgtaaagggcgcgtaggcggatttttaagtctggtgtgaaagatcagggctcaaccctgagagtgcatcggaaactggagatcttgaggacaggagaggaaagtggaattccacgtgtagcggtgaaatgcgtagatatgtggaggaacaccagtggcgaaggcgactttctggactgtaactgacgctgaggcgcgaaagcgtggggagcaaacaggattagataccctggtagtccacgctgtaaacgatgagtgctaggtgtagagggtatcgaccccttctgtgccgcagttaacacaataagcactccgcctggggagtacggccgcaaggttgaaactcaaaggaattgacgggggcccgcacaagcggtggagcatgtggtttaattcgacgcaacgcgaagaaccttaccaaggcttgacatccacagaatcctaaggaaacttgggagtgcccttcggggagctgtgagacaggtggtgcatggttgtcgtcagctcgtgtcgtgagatgttgggttaagtcccgcaacgagcgcaacccctgtgtttagttgctaacgcgtaatggcgagcactctagacagactgccggtgataaaccggaggaaggtggggatgacgtcaaatcatcatgccccttatgtcttgggctacacacgtgctacaatggccggtacagacggaagcgaagccgcgaggtgaagccaatccgagaaagccggtctcagttcggattgcaggctgcaactcgcctgcatgaagtcggaatcgctagtaatcgcaggtcagcatactgcggtgaatacgttcccgggccttgtacacaccgcccgtcacaccacgaaagtctgcaacacccgaagccggtgaggtaacccgaaagggagctagccgtcgaaggtggggccgatgattggggtgaagtcgtaacaaggtagccgtatcggaaggtgcggctggatcacctcctt